European Patent Specification EP 3 874 056 B1, published June 14, 2023. Title: Enzymatic method for preparation of UDP-GlcNAc. Applicant: Max-Planck-Gesellschaft zur Foerderung der Wissenschaften e.V. The sequence listing filed with the application follows.

SEQUENCE LISTING (10 sequences)

SEQ ID NO: 1 - protein, 359 aa, Bifido-bacterium longum
  PEPTIDE (1)..(359): N-acetylhexosamine 1-kinase
MTESNEDLFGIASHFALEGAVTGIEPYGDGHINTTYLVTTDGPRYILQQMNTSIFPDTVNLMRNVELVTSTLKAQGKETLDIVPTTSGATWAEIDGGAWRVYKFIEHTVSYNLVPNPDVFREAGSAFGDFQNFLSEFDASQLTETIAHFHDTPHRFEDFKAALAADKLGRAAACQPEIDFYLSHADQYAVVMDGLRDGSIPLRVTHNDTKLNNILMDATTGKARAIIDLDTIMPGSMLFDFGDSIRFGASTALEDEKDLSKVHFSTELFRAYTEGFVGELRGSITAREAELLPFSGNLLTMECGMRFLADYLEGDIYFATKYPEHNLVRTRTQIKLVQEMEQKASETRAIVADIMEAAR

SEQ ID NO: 2 - protein, 202 aa, Arabidopsis thaliana [sequence omitted]

SEQ ID NO: 3 - protein, 301 aa, Ruegeria pomeroyi
  PEPTIDE (1)..(301): polyphosphate kinase 3
MNRNGSTKDPRRMTGAATGEISRYFNDKAPKDIRRAIEKADKDDILSTTYPYDAEMTAKDYRAQMEALQIELVKLQAWIKQSGARVALLFEGRDAAGKGGTIKRFRENLNPRGARVVALSKPTEAERSQWYFQRYIQHLPSAGELVFYDRSWYNRGVVEHVFGWCDEEQRERFFRQVMPFEHDLVDDGIHLFKFWLNVGRAEQLRRFHDRERDPLKQWKLSPVDIAGLDKWEAYTTAISQTLTRSHSDRAPWTVIRSDDKKRARLAAIRTVLSGIDYDNKDRAAVGQPDAAICGGPDIWDA

SEQ ID NO: 4 - protein, 302 aa, E. coli K-12 MG1655
  PEPTIDE (1)..(302): glucose 1-phosphate uridylyltransferase
MAAINTKVKKAVIPVAGLGTRMLPATKAIPKEMLPLVDKPLIQYVVNECIAAGITEIVLVTHSSKNSIENHFDTSFELEAMLEKRVKRQLLDEVQSICPPHVTIMQVRQGLAKGLGHAVLCAHPVVGDEPVAVILPDVILDEYESDLSQDNLAEMIRRFDETGHSQIMVEPVADVTAYGVVDCKGVELAPGESVPMVGVVEKPKADVAPSNLAIVGRYVLSADIWPLLAKTPPGAGDEIQLTDAIDMLIEKETVEAYHMKGKSHDCGNKLGYMQAFVEYGIRHNTLGTEFKAWLEEEMGIKK

SEQ ID NO: 5 - protein, 175 aa, Pasteurella multocida subsp. multocida str. Pm70
  PEPTIDE (1)..(175): inorganic diphosphatase
MGLETVPAGKALPDDIYVVIEIPANSDPIKYEVDKESGALFVDRFMATAMFYPANYGYVNNTLSLDGDPVDVLVPTPYPLQPGSVIRCRPVGVLKMTDEAGSDAKVVAVPHSKLTKEYDHIKDVNDLPALLKAQIQHFFESYKALEAGKWVKVDGWEGVDAARQEILDSFERAKK

SEQ ID NO: 6 - protein, 304 aa, Pseudomonas aeruginosa
  PEPTIDE (1)..(304): 1-domain polyphosphate kinase 2
MDSYGDTSGRIGRDWLDRHDEELEQELLDDELNLDELFGPEQEDAPGELSRRRYFRELFRLQRELVKLQNWVVHTGHKVVILFEGRDAAGKGGVIKRITQRLNPRVCRVAALPAPNDREQTQWYFQRYVSHLPAGGEIVLFDRSWYNRAGVERVMGFCNDEQYEEFFRSVPEFEKMLARSGIQLLKYWFSISDAEQHLRFLSRIHDPLKQWKLSPMDLESRRRWEAYTKAKETMLERTHIPEAPWWVVQADDKKRARLNCIHHLLQQMPYREVPQPPVHLPERLRHADYVRHPTPGEIIVPEVY

SEQ ID NO: 7 - protein, 496 aa, Pseudomonas aeruginosa
  PEPTIDE (1)..(496): 2-domain polyphosphate kinase 2
MFESAEVGHSIDKDTYEKAVIELREALLEAQFELKQQARFPVIILINGIEGAGKGETVKLLNEWMDPRLIEVQSFLRPSDEELERPPQWRFWRRLPPKGRTGIFFGNWYSQMLYARVEGHIKEAKLDQAIDAAERFERMLCDEGALLFKFWFHLSKKQLKERLKALEKDPQHSWKLSPLDWKQSEVYDRFVHYGERVLRRTSRDYAPWYVVEGADERYRALTVGRILLEGLQAALATKERAKRQPHAAPLVSSLDNRGLLDSLDLGQYLDKDAYKEQLAAEQARLAGLIRDKRFRQHSLVAVFEGNDAAGKGGAIRRVTDALDPRQYHIVPIAAPTEEERAQPYLWRFWRHIPARRQFTIFDRSWYGRVLVERIEGFCAPADWLRAYGEINDFEEQLSEYGIIVVKFWLAIDKQTQMERFKEREKTPYKRYKITEEDWRNRDKWDQYVDAVGDMVDRTSTEIAPWTLVEANDKRFARVKVLRTINDAIEAAYKKDK

SEQ ID NO: 8 - protein, 458 aa, Pasteurella multocida
  PEPTIDE (1)..(458): UTP-GlcNAc-1-phosphate uridylyltransferase
MKEKALSIVILAAGKGTRMYSDLPKVLHKIAGKPMVKHVIDTVKSIHAKNIHLVYGHGGEVMQTRLQDEPVNWVLQAEQLGTGHAMQQAAPFFADDENILMLYGDGPLITAETLQTLIAAKPEHGIALLTVVLDDPTGYGRIVRENGNVVAIVEQKDANAEQLKIQEINTGLLVADGKSLKKWLSQLTNNNAQGEYYITDVIALANQDGCQVVAVQASDFMEVEGVNNRQQLARLERYYQRKQADNLLLAGVALADPERFDLRGELSHGKDVEIDVNVIIEGKVSLGHRVKIGAGCVLKNCQIGDDVEIKPYSVLEEAIVGQAAQIGPFSRLRPGTALADNTHIGNFVEIKKAHIGTGSKVNHLSYVGDAEVGMQCNIGAGVITCNYDGANKFKTIIGDNVFVGSDVQLVAPVTIETGATIGAGTTVTKDVACDELVISRVPQRHIQGWQRPTKQTKK

SEQ ID NO: 9 - protein, 213 aa, Escherichia coli
  PEPTIDE (1)..(213): uridine/cytidine kinase
MTDQSHQCVIIGIAGASASGKSLIASTLYRELREQVGDEHIGVIPEDCYYKDQSHLSMEERVKTNYDHPSAMDHSLLLEHLQALKRGSAIDLPVYSYVEHTRMKETVTVEPKKVIILEGILLLTDARLRDELNFSIFVDTPLDICLMRRIKRDVNERGRSMDSVMAQYQKTVRPMFLQFIEPSKQYADIIVPRGGKNRIAIDILKAKISQFFE

SEQ ID NO: 10 - protein, 333 aa, Escherichia coli
  PEPTIDE (1)..(333): beta-1,3-N-acetylglucosamine transferase
MQPLVSVLICAYNVEKYFAQSLAAVVNQTWRNLDILIVDDGSTDGTLAIAQRFQEQDGRIRILAQPRNSGLIPSLNIGLDELAKSGGGGEYIARTDADDIAAPDWIEKIVGEMEKDRSIIAMGAWLEVLSEEKDGNRLARHHEHGKIWKKPTRHEDIADFFPFGNPIHNNTMIMRRSVIDGGLRYNTERDWAEDYQFWYDVSKLGRLAYYPEALVKYRLHANQVSSKYSIRQHEIAQGIQKTARNDFLQSMGFKTRFDSLEYRQIKAVAYELLEKHLPEEDFELARRFLYQCFKRTDTLPAGAWLDFAADGRMRRLFTLRQYFGILHRLLKNR